European Patent Application EP 4 706 675 A1, published March 11, 2026. Title: Cysteine-engineered Chimeric Antigen Receptor. Applicant: Max-Planck-Gesellschaft zur Förderung der Wissenschaften e.V. The sequence listing filed with the application follows.

SEQUENCE LISTING (61 sequences)

SEQ ID NO: 1 - protein, 245 aa, synthetic construct
DIQMTQTTSSLSASLGDRVTISCRASQDISKYLNWYQQKPDGTVKLLIYHTSRLHSGVPSRFSGSGSGTDYSLTISNLEQEDIATYFCQQGNTLPYTFGGGTKLEITGSTSGSGKPGSGEGSTKGEVKLQESGPGLVAPSQSLSVTCTVSGVSLPDYGVSWIRQPPRKGLEWLGVIWGSETTYYNSALKSRLTIIKDNSKSQVFLKMNSLQTDDTAIYYCAKHYYYGGSYAMDYWGQGTSVTVSS

SEQ ID NO: 2 - protein, 245 aa, synthetic construct
DIQMTQTTSSLSASLGDRVTISCRASQDISKYLNWYQQKPDGTVKLLIYHTSRLHSGVPSRFSGSGSGTDYSLTISNLEQEDIATYFCQQGNTLPYTFGGGTKLEITGSTSGSGKPGSGEGSTKGEVKLQESGPGLVAPSQSLSVTCTVSGVSLPDYGVSWIRQPPRKGLEWLGVIWGSETTYYNSALKSRLTIIKDNSKSQVFLKMNSLQTDDTAIYYCAKHYYYGGCYAMDYWGQGTSVTVSS

SEQ ID NO: 3 - protein, 245 aa, synthetic construct
DIQMTQTTSSLSASLGDRVTISCRASQDISKYLNWYQQKPDGTVKLLIYHTSRLHSGVPSRFSGSGSGTDYSLTISNLEQEDIATYFCQQGNTLPYTFGGGTKLEITGSTSGSGKPGSGEGSTKGEVKLQESGPGLVAPSQSLSVTCTVSGVSLPDYGVSWIRQPPRKGLEWLGVIWGSETTYYNSALKSRLTIIKDNSKSQVFLKMNSLQTDDTAIYYCAKHYYYGCSYAMDYWGQGTSVTVSS

SEQ ID NO: 4 - protein, 245 aa, synthetic construct
DIQMTQTTSSLSASLGDRVTISCRASQDISKYLNWYQQKPDGTVKLLIYHTSRLHSGVPSRFSGSGSGTDYSLTISNLEQEDIATYFCQQGCTLPYTFGGGTKLEITGSTSGSGKPGSGEGSTKGEVKLQESGPGLVAPSQSLSVTCTVSGVSLPDYGVSWIRQPPRKGLEWLGVIWGSETTYYNSALKSRLTIIKDNSKSQVFLKMNSLQTDDTAIYYCAKHYYYGGSYAMDYWGQGTSVTVSS

SEQ ID NO: 5 - protein, 123 aa, synthetic construct
GHVQLVESGGGLVQPGGSLRLSCAASGFTFSNYRMYWIRQAPGKGLEWVSTISSDGVATYYADSVKGRFTISRDNAKNTLYLQMNRLKLEDTAVYSCAALNRYCGNEYEYDYRGQGTQVTVSS

SEQ ID NO: 6 - protein, 127 aa, synthetic construct
QVQLVESGGRLVQAGDSLRLSCAASGRTFSTSAMAWFRQAPGREREFVAAITWTVGNTILGDSVKGRFTISRDRAKNTVDLQMDNLEPEDTAVYYCSARSRGYVLSVLRSVDSYDYWGQGTQVTVSS

SEQ ID NO: 7 - protein, 45 aa, synthetic construct
TTTPAPRPPTPAPTIASQPLSLRPEACRPAAGGAVHTRGLDFACD

SEQ ID NO: 8 - protein, 232 aa, synthetic construct
EPKSCDKTHTCPPCPAPELLGGPSVFLFPPKPKDTLMISRTPEVTCVVVDVSHEDPEVKFNWYVDGVEVHNAKTKPREEQYNSTYRVVSVLTVLHQDWLNGKEYKCKVSNKALPAPIEKTISKAKGQPREPQVYTLPPSRDELTKNQVSLTCLVKGFYPSDIAVEWESNGQPENNYKTTPPVLDSDGSFFLYSKLTVDKSRWQQGNVFSCSVMHEALHNHYTQKSLSLSPVD

SEQ ID NO: 9 - protein, 24 aa, synthetic construct
IYIWAPLAGTCGVLLLSLVITLYC

SEQ ID NO: 10 - protein, 43 aa, synthetic construct
GSRSKRSRLLHSDYMNMTPRRPGPTRKHYQPYAPPRDFAAYRS

SEQ ID NO: 11 - protein, 43 aa, synthetic construct; identical to SEQ ID NO: 10

SEQ ID NO: 12 - protein, 42 aa, synthetic construct
KRGRKKLLYIFKQPFMRPVQTTQEEDGCSCRFPEEEEGGCEL

SEQ ID NO: 13 - protein, 112 aa, synthetic construct
RVKFSRSADAPAYQQGQNQLYNELNLGRREEYDVLDKRRGRDPEMGGKPRRKNPQEGLYNELQKDKMAEAYSEIGMKGERRRGKGHDGLYQGLSTATKDTYDALHMQALPPR

SEQ ID NO: 14 - protein, 21 aa, synthetic construct
MALPVTALLLPLALLLHAARP

SEQ ID NO: 15 - protein, 22 aa, synthetic construct
MLLLVTSLLLCELPHPAFLLIP

SEQ ID NO: 16 - DNA, 735 bp, synthetic construct
  source 1..735: mol_type = other DNA
gacatccagatgacccagaccacaagcagcctgtctgccagcctgggcgatagagtgaccatcagctgtagagccagccaggacatcagcaagtacctgaactggtatcagcaaaagcccgacggcaccgtgaagctgctgatctaccacaccagcagactgcacagcggcgtgccaagcagattttctggcagcggctctggcaccgactacagcctgacaatcagcaacctggaacaagaggatatcgctacctacttctgccagcaaggcaacaccctgccttacacctttggcggaggcaccaagctggaaatcaccggctctacaagcggcagcggcaaacctggatctggcgagggatctaccaagggcgaagtgaaactgcaagagtctggccctggactggtggccccatctcagtctctgagcgtgacctgtacagtcagcggagtgtccctgcctgattacggcgtgtcctggatcagacagcctcctcggaaaggcctggaatggctgggagtgatctggggcagcgagacaacctactacaacagcgccctgaagtcccggctgaccatcatcaaggacaactccaagagccaggtgttcctgaagatgaacagcctgcagaccgacgacaccgccatctactattgcgccaagcactactactacggcggcagctacgccatggattattggggccagggcaccagcgtgacagtttcttca

SEQ ID NO: 17 - DNA, 369 bp, synthetic construct
  source 1..369: mol_type = other DNA
ggccacgtgcagctggtggagagcggcggcggcctggtgcagcccggcggcagcctgcgcctgagctgcgccgccagcggcttcaccttcagcaactaccgcatgtactggatacgccaggcccccggcaagggcctggagtgggtgagcaccatcagcagcgacggcgtggccacctactacgccgacagcgtgaagggccgcttcaccatcagccgcgacaacgccaagaacaccctgtacctgcagatgaaccgcctgaagctggaggacaccgccgtgtacagctgcgccgccctgaaccgctactgcggcaacgagtacgagtacgactaccgcggccagggcacccaggtgaccgtgagcagc

SEQ ID NO: 18 - DNA, 388 bp, synthetic construct
  source 1..388: mol_type = other DNA
caagttcaactggtggaaagtggcgggagacttgtgcaggccggcgatagcctgcggctctcatgtgcagcctctggcagaactttctccacgtcagccatggcctggtttagacaagctccaggaagggagcgggaatttgtggccgcgattacctggactgtcgggaacactatcctgggagattcagttaagggccgctttaccatatcccgggatcgggctaagaataccgtggacctccagatggacaaccttgagcctgaagacaccgcagtctactactgtgctgtccgtgctgcggagccgcggctacgtactttgcgtgctgcgctctgtggacagctacgattactggggacagggcacacaagtgacagtcagctct

SEQ ID NO: 19 - DNA, 135 bp, synthetic construct
  source 1..135: mol_type = other DNA
acaacaacaccagctcctcggcctccaactcctgctcctacaattgcctctcagcctctgtctctgaggcccgaagcttgtagacctgctgctggcggagctgtgcacaccagaggactggatttcgcctgcgac

SEQ ID NO: 20 - DNA, 696 bp, synthetic construct
  source 1..696: mol_type = other DNA
gagcccaaatcttgtgacaaaactcacacatgcccaccgtgcccagcacctgaactcctggggggaccgtcagtcttcctcttccccccaaaacccaaggacaccctcatgatctcccggacccctgaggtcacatgcgtggtggtggacgtgagccacgaagaccctgaggtcaagttcaactggtacgtggacggcgtggaggtgcataatgccaagacaaagccgcgggaggagcagtacaacagcacgtaccgtgtggtcagcgtcctcaccgtcctgcaccaggactggctgaatggcaaggagtacaagtgcaaggtctccaacaaagccctcccagcccccatcgagaaaaccatctccaaagccaaagggcagccccgagaaccacaggtgtacaccctgcccccatcccgggatgagctgaccaagaaccaggtcagcctgacctgcctggtcaaaggcttctatcccagcgacatcgccgtggagtgggagagcaatgggcagccggagaacaactacaagaccacgcctcccgtgctggactccgacggctccttcttcctctacagcaagctcaccgtggacaagagcaggtggcagcaggggaacgtcttctcatgctccgtgatgcatgaggctctgcacaaccactacacacagaagagcctctccctgtctccggtcgac

SEQ ID NO: 21 - DNA, 72 bp, synthetic construct
  source 1..72: mol_type = other DNA
atctacatttgggcccctctggctggaacatgcggagttctgctgctgagcctggtcatcaccctgtactgc

SEQ ID NO: 22 - DNA, 81 bp, synthetic construct
  source 1..81: mol_type = other DNA
ttttgggtgctggtggtggttggtggagtcctggcttgctatagcttgctagtaacagtggcctttattattttctgggtg

SEQ ID NO: 23 - DNA, 129 bp, synthetic construct
  source 1..129: mol_type = other DNA
ggatccaggagtaagaggagcaggctcctgcacagtgactacatgaacatgactccccgccgccccgggcccacccgcaagcattaccagccctatgccccaccacgcgacttcgcagcctatcgctcc

SEQ ID NO: 24 - DNA, 126 bp, synthetic construct
  source 1..126: mol_type = other DNA
aagcggggcagaaagaagctgctgtacatcttcaagcagcccttcatgcggcccgtgcagaccacacaagaggaagatggctgctcctgcagattccccgaggaagaagaaggcggctgcgagctg

SEQ ID NO: 25 - DNA, 336 bp, synthetic construct
  source 1..336: mol_type = other DNA
agagtgaagttctccagatctgccgacgctcctgcctaccagcagggccagaatcagctgtacaacgagctgaacctggggagaagagaagagtacgacgtgctggataagcggagaggcagagatcctgagatgggcggcaagcccagacggaagaatcctcaagagggcctgtataatgagctgcagaaagacaagatggccgaggcctacagcgagatcggaatgaagggcgagcgcagaagaggcaagggccacgatggactgtatcagggcctgagcacagccaccaaggatacctatgatgccctgcacatgcaggccctgcctccaaga

SEQ ID NO: 26 - DNA, 63 bp, synthetic construct
  source 1..63: mol_type = other DNA
atggccttaccagtgaccgccttgctcctgccgctggccttgctgctccacgccgccaggccg

SEQ ID NO: 27 - DNA, 66 bp, synthetic construct
  source 1..66: mol_type = other DNA
atgctgctgctggtcacatctctgctgctgtgcgagctgccccatcctgcctttctgctgatcccc

SEQ ID NO: 28 - RNA, 735 nt, synthetic construct
  source 1..735: mol_type = other RNA
gacatccagatgacccagaccacaagcagcctgtctgccagcctgggcgatagagtgaccatcagctgtagagccagccaggacatcagcaagtacctgaactggtatcagcaaaagcccgacggcaccgtgaagctgctgatctaccacaccagcagactgcacagcggcgtgccaagcagattttctggcagcggctctggcaccgactacagcctgacaatcagcaacctggaacaagaggatatcgctacctacttctgccagcaaggcaacaccctgccttacacctttggcggaggcaccaagctggaaatcaccggctctacaagcggcagcggcaaacctggatctggcgagggatctaccaagggcgaagtgaaactgcaagagtctggccctggactggtggccccatctcagtctctgagcgtgacctgtacagtcagcggagtgtccctgcctgattacggcgtgtcctggatcagacagcctcctcggaaaggcctggaatggctgggagtgatctggggcagcgagacaacctactacaacagcgccctgaagtcccggctgaccatcatcaaggacaactccaagagccaggtgttcctgaagatgaacagcctgcagaccgacgacaccgccatctactattgcgccaagcactactactacggcggcagctacgccatggattattggggccagggcaccagcgtgacagtttcttca

SEQ ID NO: 29 - RNA, 369 nt, synthetic construct
  source 1..369: mol_type = other RNA
ggccacgtgcagctggtggagagcggcggcggcctggtgcagcccggcggcagcctgcgcctgagctgcgccgccagcggcttcaccttcagcaactaccgcatgtactggatacgccaggcccccggcaagggcctggagtgggtgagcaccatcagcagcgacggcgtggccacctactacgccgacagcgtgaagggccgcttcaccatcagccgcgacaacgccaagaacaccctgtacctgcagatgaaccgcctgaagctggaggacaccgccgtgtacagctgcgccgccctgaaccgctactgcggcaacgagtacgagtacgactaccgcggccagggcacccaggtgaccgtgagcagc

SEQ ID NO: 30 - RNA, 381 nt, synthetic construct
  source 1..381: mol_type = other RNA
caagttcaactggtggaaagtggcgggagacttgtgcaggccggcgatagcctgcggctctcatgtgcagcctctggcagaactttctccacgtcagccatggcctggtttagacaagctccaggaagggagcgggaatttgtggccgcgattacctggactgtcgggaacactatcctgggagattcagttaagggccgctttaccatatcccgggatcgggctaagaataccgtggacctccagatggacaaccttgagcctgaagacaccgcagtctactactgttctgctcggagccgcggctacgtacttagtgtgctgcgctctgtggacagctacgattactggggacagggcacacaagtgacagtcagctct

SEQ ID NO: 31 - RNA, 135 nt, synthetic construct
  source 1..135: mol_type = other RNA
acaacaacaccagctcctcggcctccaactcctgctcctacaattgcctctcagcctctgtctctgaggcccgaagcttgtagacctgctgctggcggagctgtgcacaccagaggactggatttcgcctgcgac

SEQ ID NO: 32 - RNA, 696 nt, synthetic construct
  source 1..696: mol_type = other RNA
gagcccaaatcttgtgacaaaactcacacatgcccaccgtgcccagcacctgaactcctggggggaccgtcagtcttcctcttccccccaaaacccaaggacaccctcatgatctcccggacccctgaggtcacatgcgtggtggtggacgtgagccacgaagaccctgaggtcaagttcaactggtacgtggacggcgtggaggtgcataatgccaagacaaagccgcgggaggagcagtacaacagcacgtaccgtgtggtcagcgtcctcaccgtcctgcaccaggactggctgaatggcaaggagtacaagtgcaaggtctccaacaaagccctcccagcccccatcgagaaaaccatctccaaagccaaagggcagccccgagaaccacaggtgtacaccctgcccccatcccgggatgagctgaccaagaaccaggtcagcctgacctgcctggtcaaaggcttctatcccagcgacatcgccgtggagtgggagagcaatgggcagccggagaacaactacaagaccacgcctcccgtgctggactccgacggctccttcttcctctacagcaagctcaccgtggacaagagcaggtggcagcaggggaacgtcttctcatgctccgtgatgcatgaggctctgcacaaccactacacacagaagagcctctccctgtctccggtcgac

SEQ ID NO: 33 - RNA, 72 nt, synthetic construct
  source 1..72: mol_type = other RNA
atctacatttgggcccctctggctggaacatgcggagttctgctgctgagcctggtcatcaccctgtactgc

SEQ ID NO: 34 - RNA, 81 nt, synthetic construct
  source 1..81: mol_type = other RNA
ttttgggtgctggtggtggttggtggagtcctggcttgctatagcttgctagtaacagtggcctttattattttctgggtg

SEQ ID NO: 35 - RNA, 129 nt, synthetic construct
  source 1..129: mol_type = other RNA
ggatccaggagtaagaggagcaggctcctgcacagtgactacatgaacatgactccccgccgccccgggcccacccgcaagcattaccagccctatgccccaccacgcgacttcgcagcctatcgctcc

SEQ ID NO: 36 - RNA, 126 nt, synthetic construct
  source 1..126: mol_type = other RNA
aagcggggcagaaagaagctgctgtacatcttcaagcagcccttcatgcggcccgtgcagaccacacaagaggaagatggctgctcctgcagattccccgaggaagaagaaggcggctgcgagctg

SEQ ID NO: 37 - RNA, 336 nt, synthetic construct
  source 1..336: mol_type = other RNA
agagtgaagttctccagatctgccgacgctcctgcctaccagcagggccagaatcagctgtacaacgagctgaacctggggagaagagaagagtacgacgtgctggataagcggagaggcagagatcctgagatgggcggcaagcccagacggaagaatcctcaagagggcctgtataatgagctgcagaaagacaagatggccgaggcctacagcgagatcggaatgaagggcgagcgcagaagaggcaagggccacgatggactgtatcagggcctgagcacagccaccaaggatacctatgatgccctgcacatgcaggccctgcctccaaga

SEQ ID NO: 38 - RNA, 63 nt, synthetic construct
  source 1..63: mol_type = other RNA
atggccttaccagtgaccgccttgctcctgccgctggccttgctgctccacgccgccaggccg

SEQ ID NO: 39 - RNA, 66 nt, synthetic construct
  source 1..66: mol_type = other RNA
atgctgctgctggtcacatctctgctgctgtgcgagctgccccatcctgcctttctgctgatcccc

SEQ ID NO: 40 - protein, 242 aa, synthetic construct
EVQLLQSGPELEKPGASVMISCKASGSSFTGYNMNWVRQNIGKSLEWIGAIDPYYGGTSYNQKFKGRATLTVDKSSSTAYMHLKSLTSEDSAVYYCVSGMEYWGQGTSVTVSSGGGGSGGGGSGGGGSEIVMTQSPATLSVSPGERATLSCRSSQSLVHRNGNTYLHWYLQKPGQSPKLLIHKVSNRFSGVPDRFSGSGSGTDFTLKISRVEAEDLGVYFCSQSTHVPPLTFGAGTKLELKR

SEQ ID NO: 41 - protein, 242 aa, synthetic construct
EVQLLQSGPELEKPGASVMISCKASGSSFTGYNMNWVRQNIGKSLEWIGAIDPYYGGTSYNQKFKGRATLTVDKSSSTAYMHLKSLTSEDSAVYYCVSGCEYWGQGTSVTVSSGGGGSGGGGSGGGGSEIVMTQSPATLSVSPGERATLSCRSSQSLVHRNGNTYLHWYLQKPGQSPKLLIHKVSNRFSGVPDRFSGSGSGTDFTLKISRVEAEDLGVYFCSQSTHVPPLTFGAGTKLELKR

SEQ ID NO: 42 - protein, 242 aa, synthetic construct
EVQLLQSGPELEKPGASVMISCKASGSSFTGYNMNWVRQNIGKSLEWIGAIDPYYGGTSYNQKFKGRATLTVDKSSSTAYMHLKSLTSEDSAVYYCVSGMEYWGQGTSVTVSSGGGGSGGGGSGGGGSEIVMTQSPATLSVSPGERATLSCRSSQSLVHRNGNTYLHWYLQKPGQSPKLLIHKVSNRFSGVPDRFSGSGSGTDFTLKISRVEAEDLGVYFCSQSTCVPPLTFGAGTKLELKR

SEQ ID NO: 43 - protein, 242 aa, synthetic construct
EVQLLQSGPELEKPGASVMISCKASGSSFTGYNMNWVRQNIGKSLEWIGAIDPYYGGTSYNQKFKGRATLTVDKSSSTAYMHLKSLTSEDSAVYYCVSGMEYWGQGTSVTVSSGGGGSGGGGSGGGGSEIVMTQSPATLSVSPGERATLSCRSSQSLVHRNGNTYLHWYLQKPGQSPKLLIHKVSNRFSGVPDRFSGSGSGTDFTLKISRVEAEDLGVYFCSQSTHCPPLTFGAGTKLELKR

SEQ ID NO: 44 - DNA, 726 bp, synthetic construct
  source 1..726: mol_type = other DNA
gaagtgcagctgctgcagtctggccctgaactggaaaaacctggcgcctccgtgatgatcagctgtaaagccagcggcagcagcttcaccggctacaacatgaactgggtccgacagaacatcggcaagagcctggaatggatcggcgccatcgatccttactacggcggcaccagctacaaccagaagttcaagggcagagccacactgaccgtggacaagagcagcagcacagcctacatgcacctgaagtccctgacaagcgaggacagcgccgtgtactactgtgtgtccggcatggaatattggggccagggcacaagcgtgacagtttcttctggtggcggaggatctggcggaggtggaagcggcggaggcggatctgaaatcgtgatgacacagagccccgccactctgagtgtgtctccaggcgaaagagctaccctgagctgtagaagcagccagagcctggtgcacagaaacggcaatacctacctgcactggtatctgcagaagcccggccagtctcctaagctgctgatccacaaggtgtccaacagattcagcggcgtgcccgatagattttctggctctggcagcggcaccgacttcaccctgaagattagcagagtggaagccgaggacctgggcgtgtacttctgtagccagtctacacacgtgccacctctgacctttggcgctggcacaaagctggaactgaagcgg

SEQ ID NO: 45 - DNA, 726 bp, synthetic construct
  source 1..726: mol_type = other DNA
gaagtgcagctgctgcagtctggccctgaactggaaaaacctggcgcctccgtgatgatcagctgtaaagccagcggcagcagcttcaccggctacaacatgaactgggtccgacagaacatcggcaagagcctggaatggatcggcgccatcgatccttactacggcggcaccagctacaaccagaagttcaagggcagagccacactgaccgtggacaagagcagcagcacagcctacatgcacctgaagtccctgacaagcgaggacagcgccgtgtactactgtgtgtccggctgtgaatattggggccagggcacaagcgtgacagtttcttctggtggcggaggatctggcggaggtggaagcggcggaggcggatctgaaatcgtgatgacacagagccccgccactctgagtgtgtctccaggcgaaagagctaccctgagctgtagaagcagccagagcctggtgcacagaaacggcaatacctacctgcactggtatctgcagaagcccggccagtctcctaagctgctgatccacaaggtgtccaacagattcagcggcgtgcccgatagattttctggctctggcagcggcaccgacttcaccctgaagattagcagagtggaagccgaggacctgggcgtgtacttctgtagccagtctacacacgtgccacctctgacctttggcgctggcacaaagctggaactgaagcgg

SEQ ID NO: 46 - DNA, 726 bp, synthetic construct
  source 1..726: mol_type = other DNA
gaagtgcagctgctgcagtctggccctgaactggaaaaacctggcgcctccgtgatgatcagctgtaaagccagcggcagcagcttcaccggctacaacatgaactgggtccgacagaacatcggcaagagcctggaatggatcggcgccatcgatccttactacggcggcaccagctacaaccagaagttcaagggcagagccacactgaccgtggacaagagcagcagcacagcctacatgcacctgaagtccctgacaagcgaggacagcgccgtgtactactgtgtgtccggcatggaatattggggccagggcacaagcgtgacagtttcttctggtggcggaggatctggcggaggtggaagcggcggaggcggatctgaaatcgtgatgacacagagccccgccactctgagtgtgtctccaggcgaaagagctaccctgagctgtagaagcagccagagcctggtgcacagaaacggcaatacctacctgcactggtatctgcagaagcccggccagtctcctaagctgctgatccacaaggtgtccaacagattcagcggcgtgcccgatagattttctggctctggcagcggcaccgacttcaccctgaagattagcagagtggaagccgaggacctgggcgtgtacttctgtagccagtctacatgtgtgccacctctgacctttggcgctggcacaaagctggaactgaagcgg

SEQ ID NO: 47 - DNA, 726 bp, synthetic construct
  source 1..726: mol_type = other DNA
gaagtgcagctgctgcagtctggccctgaactggaaaaacctggcgcctccgtgatgatcagctgtaaagccagcggcagcagcttcaccggctacaacatgaactgggtccgacagaacatcggcaagagcctggaatggatcggcgccatcgatccttactacggcggcaccagctacaaccagaagttcaagggcagagccacactgaccgtggacaagagcagcagcacagcctacatgcacctgaagtccctgacaagcgaggacagcgccgtgtactactgtgtgtccggcatggaatattggggccagggcacaagcgtgacagtttcttctggtggcggaggatctggcggaggtggaagcggcggaggcggatctgaaatcgtgatgacacagagccccgccactctgagtgtgtctccaggcgaaagagctaccctgagctgtagaagcagccagagcctggtgcacagaaacggcaatacctacctgcactggtatctgcagaagcccggccagtctcctaagctgctgatccacaaggtgtccaacagattcagcggcgtgcccgatagattttctggctctggcagcggcaccgacttcaccctgaagattagcagagtggaagccgaggacctgggcgtgtacttctgtagccagtctacacactgtccacctctgacctttggcgctggcacaaagctggaactgaagcgg

SEQ ID NO: 48 - RNA, 726 nt, synthetic construct
  source 1..726: mol_type = other RNA
gaagtgcagctgctgcagtctggccctgaactggaaaaacctggcgcctccgtgatgatcagctgtaaagccagcggcagcagcttcaccggctacaacatgaactgggtccgacagaacatcggcaagagcctggaatggatcggcgccatcgatccttactacggcggcaccagctacaaccagaagttcaagggcagagccacactgaccgtggacaagagcagcagcacagcctacatgcacctgaagtccctgacaagcgaggacagcgccgtgtactactgtgtgtccggcatggaatattggggccagggcacaagcgtgacagtttcttctggtggcggaggatctggcggaggtggaagcggcggaggcggatctgaaatcgtgatgacacagagccccgccactctgagtgtgtctccaggcgaaagagctaccctgagctgtagaagcagccagagcctggtgcacagaaacggcaatacctacctgcactggtatctgcagaagcccggccagtctcctaagctgctgatccacaaggtgtccaacagattcagcggcgtgcccgatagattttctggctctggcagcggcaccgacttcaccctgaagattagcagagtggaagccgaggacctgggcgtgtacttctgtagccagtctacacacgtgccacctctgacctttggcgctggcacaaagctggaactgaagcgg

SEQ ID NO: 49 - RNA, 726 nt, synthetic construct
  source 1..726: mol_type = other RNA
gaagtgcagctgctgcagtctggccctgaactggaaaaacctggcgcctccgtgatgatcagctgtaaagccagcggcagcagcttcaccggctacaacatgaactgggtccgacagaacatcggcaagagcctggaatggatcggcgccatcgatccttactacggcggcaccagctacaaccagaagttcaagggcagagccacactgaccgtggacaagagcagcagcacagcctacatgcacctgaagtccctgacaagcgaggacagcgccgtgtactactgtgtgtccggctgtgaatattggggccagggcacaagcgtgacagtttcttctggtggcggaggatctggcggaggtggaagcggcggaggcggatctgaaatcgtgatgacacagagccccgccactctgagtgtgtctccaggcgaaagagctaccctgagctgtagaagcagccagagcctggtgcacagaaacggcaatacctacctgcactggtatctgcagaagcccggccagtctcctaagctgctgatccacaaggtgtccaacagattcagcggcgtgcccgatagattttctggctctggcagcggcaccgacttcaccctgaagattagcagagtggaagccgaggacctgggcgtgtacttctgtagccagtctacacacgtgccacctctgacctttggcgctggcacaaagctggaactgaagcgg

SEQ ID NO: 50 - RNA, 726 nt, synthetic construct
  source 1..726: mol_type = other RNA
gaagtgcagctgctgcagtctggccctgaactggaaaaacctggcgcctccgtgatgatcagctgtaaagccagcggcagcagcttcaccggctacaacatgaactgggtccgacagaacatcggcaagagcctggaatggatcggcgccatcgatccttactacggcggcaccagctacaaccagaagttcaagggcagagccacactgaccgtggacaagagcagcagcacagcctacatgcacctgaagtccctgacaagcgaggacagcgccgtgtactactgtgtgtccggcatggaatattggggccagggcacaagcgtgacagtttcttctggtggcggaggatctggcggaggtggaagcggcggaggcggatctgaaatcgtgatgacacagagccccgccactctgagtgtgtctccaggcgaaagagctaccctgagctgtagaagcagccagagcctggtgcacagaaacggcaatacctacctgcactggtatctgcagaagcccggccagtctcctaagctgctgatccacaaggtgtccaacagattcagcggcgtgcccgatagattttctggctctggcagcggcaccgacttcaccctgaagattagcagagtggaagccgaggacctgggcgtgtacttctgtagccagtctacatgtgtgccacctctgacctttggcgctggcacaaagctggaactgaagcgg

SEQ ID NO: 51 - RNA, 726 nt, synthetic construct
  source 1..726: mol_type = other RNA
gaagtgcagctgctgcagtctggccctgaactggaaaaacctggcgcctccgtgatgatcagctgtaaagccagcggcagcagcttcaccggctacaacatgaactgggtccgacagaacatcggcaagagcctggaatggatcggcgccatcgatccttactacggcggcaccagctacaaccagaagttcaagggcagagccacactgaccgtggacaagagcagcagcacagcctacatgcacctgaagtccctgacaagcgaggacagcgccgtgtactactgtgtgtccggcatggaatattggggccagggcacaagcgtgacagtttcttctggtggcggaggatctggcggaggtggaagcggcggaggcggatctgaaatcgtgatgacacagagccccgccactctgagtgtgtctccaggcgaaagagctaccctgagctgtagaagcagccagagcctggtgcacagaaacggcaatacctacctgcactggtatctgcagaagcccggccagtctcctaagctgctgatccacaaggtgtccaacagattcagcggcgtgcccgatagattttctggctctggcagcggcaccgacttcaccctgaagattagcagagtggaagccgaggacctgggcgtgtacttctgtagccagtctacacactgtccacctctgacctttggcgctggcacaaagctggaactgaagcgg

SEQ ID NO: 52 - DNA, 27 bp, synthetic construct
  source 1..27: mol_type = other DNA
ttcaaagtttttttcttccatttcagg

SEQ ID NO: 53 - DNA, 27 bp, synthetic construct
  source 1..27: mol_type = other DNA
acaaattttgtaatccagaggttgatt

SEQ ID NO: 54 - DNA, 22 bp, synthetic construct
  source 1..22: mol_type = other DNA
ttattaggtaccgcggggaggc

SEQ ID NO: 55 - DNA, 15 bp, synthetic construct
  source 1..15: mol_type = other DNA
cgctacagcggcaac

SEQ ID NO: 56 - DNA, 15 bp, synthetic construct
  source 1..15: mol_type = other DNA
gttgccgctgtagcg

SEQ ID NO: 57 - DNA, 181 bp, synthetic construct
  source 1..181: mol_type = other DNA
gggtctctctggttagaccagatctgagcctgggagctctctggctaactagggaacccactgcttaagcctcaataaagcttgccttgagtgcttcaagtagtgtgtgcccgtctgttgtgtgactctggtaactagagatccctcagacccttttagtcagtgtggaaaatctctagca

SEQ ID NO: 58 - DNA, 234 bp, synthetic construct
  source 1..234: mol_type = other DNA
tggaagggctaattcactcccaacgaagacaagatctgctttttgcttgtactgggtctctctggttagaccagatctgagcctgggagctctctggctaactagggaacccactgcttaagcctcaataaagcttgccttgagtgcttcaagtagtgtgtgcccgtctgttgtgtgactctggtaactagagatccctcagacccttttagtcagtgtggaaaatctctagca

SEQ ID NO: 59 - DNA, 1179 bp, synthetic construct
  source 1..1179: mol_type = other DNA
ggctccggtgcccgtcagtgggcagagcgcacatcgcccacagtccccgagaagttggggggaggggtcggcaattgaaccggtgcctagagaaggtggcgcggggtaaactgggaaagtgatgtcgtgtactggctccgcctttttcccgagggtgggggagaaccgtatataagtgcagtagtcgccgtgaacgttctttttcgcaacgggtttgccgccagaacacaggtaagtgccgtgtgtggttcccgcgggcctggcctctttacgggttatggcccttgcgtgccttgaattacttccacctggctgcagtacgtgattcttgatcccgagcttcgggttggaagtgggtgggagagttcgaggccttgcgcttaaggagccccttcgcctcgtgcttgagttgaggcctggcctgggcgctggggccgccgcgtgcgaatctggtggcaccttcgcgcctgtctcgctgctttcgataagtctctagccatttaaaatttttgatgacctgctgcgacgctttttttctggcaagatagtcttgtaaatgcgggccaagatctgcacactggtatttcggtttttggggccgcgggcggcgacggggcccgtgcgtcccagcgcacatgttcggcgaggcggggcctgcgagcgcggccaccgagaatcggacgggggtagtctcaagctggccggcctgctctggtgcctggtctcgcgccgccgtgtatcgccccgccctgggcggcaaggctggcccggtcggcaccagttgcgtgagcggaaagatggccgcttcccggccctgctgcagggagctcaaaatggaggacgcggcgctcgggagagcgggcgggtgagtcacccacacaaaggaaaagggcctttccgtcctcagccgtcgcttcatgtgactccacggagtaccgggcgccgtccaggcacctcgattagttctcgagcttttggagtacgtcgtctttaggttggggggaggggttttatgcgatggagtttccccacactgagtgggtggagactgaagttaggccagcttggcacttgatgtaattctccttggaatttgccctttttgagtttggatcttggttcattctcaagcctcagacagtggttcaaagtttttttcttccatttcaggtgtcgtga

SEQ ID NO: 60 - DNA, 204 bp, synthetic construct
  source 1..204: mol_type = other DNA
gtgatgcggttttggcagtacatcaatgggcgtggatagcggtttgactcacggggatttccaagtctccaccccattgacgtcaatgggagtttgttttggcaccaaaatcaacgggactttccaaaatgtcgtaacaactccgccccattgacgcaaatgggcggtaggcgtgtacggtgggaggtctatataagcagagct

SEQ ID NO: 61 - DNA, 589 bp, synthetic construct
  source 1..589: mol_type = other DNA
aatcaacctctggattacaaaatttgtgaaagattgactggtattcttaactatgttgctccttttacgctatgtggatacgctgctttaatgcctttgtatcatgctattgcttcccgtatggctttcattttctcctccttgtataaatcctggttgctgtctctttatgaggagttgtggcccgttgtcaggcaacgtggcgtggtgtgcactgtgtttgctgacgcaacccccactggttggggcattgccaccacctgtcagctcctttccgggactttcgctttccccctccctattgccacggcggaactcatcgccgcctgccttgcccgctgctggacaggggctcggctgttgggcactgacaattccgtggtgttgtcggggaagctgacgtcctttccatggctgctcgcctgtgttgccacctggattctgcgcgggacgtccttctgctacgtcccttcggccctcaatccagcggaccttccttcccgcggcctgctgccggctctgcggcctcttccgcgtcttcgccttcgccctcagacgagtcggatctccctttgggccgcctccccgc